European Patent Application EP 4 714 472 A1, published March 25, 2026. Title: 一种基于超电荷蛋白的双组分原位粘合剂及其制备方法和用途. Applicant: 北京镧系生物科技有限公司. The sequence listing filed with the application follows.

SEQUENCE LISTING (5 sequences)

SEQ ID NO: 1 - protein, 145 aa, synthetic construct
VPGKGVPGKGVPGKGVPGKGVPGKGVPGKGVPGKGVPGKGVPGKGVPGVGVPGKGVPGKGVPGKGVPGKGVPGKGVPGKGVPGKGVPGKGVPGKGVPGVGVPGKGVPGKGVPGKGVPGKGVPGKGVPGKGVPGKGVPGKGVPGKG

SEQ ID NO: 2 - protein, 195 aa, synthetic construct
VPGKGVPGKGVPGKGVPGKGVPGKGVPGKGVPGKGVPGKGVPGKGVPGVGVPGKGVPGKGVPGKGVPGKGVPGKGVPGKGVPGKGVPGKGVPGKGVPGAGVPGKGVPGKGVPGKGVPGKGVPGKGVPGKGVPGKGVPGKGVPGKGVPGVGVPGKGVPGKGVPGKGVPGKGVPGKGVPGKGVPGKGVPGKGVPGKG

SEQ ID NO: 3 - protein, 395 aa, synthetic construct
VPGKGVPGKGVPGKGVPGKGVPGKGVPGKGVPGKGVPGKGVPGKGVPGVGVPGKGVPGKGVPGKGVPGKGVPGKGVPGKGVPGKGVPGKGVPGKGVPGVGVPGKGVPGKGVPGKGVPGKGVPGKGVPGKGVPGKGVPGKGVPGKGVPGVGVPGKGVPGKGVPGKGVPGKGVPGKGVPGKGVPGKGVPGKGVPGKGVPGRGVPGKGVPGKGVPGKGVPGKGVPGKGVPGKGVPGKGVPGKGVPGKGVPGVGVPGKGVPGKGVPGKGVPGKGVPGKGVPGKGVPGKGVPGKGVPGKGVPGVGVPGKGVPGKGVPGKGVPGKGVPGKGVPGKGVPGKGVPGKGVPGKGVPGVGVPGKGVPGKGVPGKGVPGKGVPGKGVPGKGVPGKGVPGKGVPGKG

SEQ ID NO: 4 - protein, 795 aa, synthetic construct
VPGKGVPGKGVPGKGVPGKGVPGKGVPGKGVPGKGVPGKGVPGKGVPGVGVPGKGVPGKGVPGKGVPGKGVPGKGVPGKGVPGKGVPGKGVPGKGVPGVGVPGKGVPGKGVPGKGVPGKGVPGKGVPGKGVPGKGVPGKGVPGKGVPGAGVPGKGVPGKGVPGKGVPGKGVPGKGVPGKGVPGKGVPGKGVPGKGVPGVGVPGKGVPGKGVPGKGVPGKGVPGKGVPGKGVPGKGVPGKGVPGKGVPGVGVPGKGVPGKGVPGKGVPGKGVPGKGVPGKGVPGKGVPGKGVPGKGVPGRGVPGKGVPGKGVPGKGVPGKGVPGKGVPGKGVPGKGVPGKGVPGKGVPGVGVPGKGVPGKGVPGKGVPGKGVPGKGVPGKGVPGKGVPGKGVPGKGVPGVGVPGKGVPGKGVPGKGVPGKGVPGKGVPGKGVPGKGVPGKGVPGKGVPGLGVPGKGVPGKGVPGKGVPGKGVPGKGVPGKGVPGKGVPGKGVPGKGVPGVGVPGKGVPGKGVPGKGVPGKGVPGKGVPGKGVPGKGVPGKGVPGKGVPGVGVPGKGVPGKGVPGKGVPGKGVPGKGVPGKGVPGKGVPGKGVPGKGVPGIGVPGKGVPGKGVPGKGVPGKGVPGKGVPGKGVPGKGVPGKGVPGKGVPGVGVPGKGVPGKGVPGKGVPGKGVPGKGVPGKGVPGKGVPGKGVPGKGVPGVGVPGKGVPGKGVPGKGVPGKGVPGKGVPGKGVPGKGVPGKGVPGKGVPGAGVPGKGVPGKGVPGKGVPGKGVPGKGVPGKGVPGKGVPGKGVPGKG

SEQ ID NO: 5 - protein, 895 aa, synthetic construct
VPGKGVPGKGVPGKGVPGKGVPGKGVPGKGVPGKGVPGKGVPGKGVPGVGVPGKGVPGKGVPGKGVPGKGVPGKGVPGKGVPGKGVPGKGVPGKGVPGVGVPGKGVPGKGVPGKGVPGKGVPGKGVPGKGVPGKGVPGKGVPGKGVPGAGVPGKGVPGKGVPGKGVPGKGVPGKGVPGKGVPGKGVPGKGVPGKGVPGVGVPGKGVPGKGVPGKGVPGKGVPGKGVPGKGVPGKGVPGKGVPGKGVPGVGVPGKGVPGKGVPGKGVPGKGVPGKGVPGKGVPGKGVPGKGVPGKGVPGLGVPGKGVPGKGVPGKGVPGKGVPGKGVPGKGVPGKGVPGKGVPGKGVPGVGVPGKGVPGKGVPGKGVPGKGVPGKGVPGKGVPGKGVPGKGVPGKGVPGVGVPGKGVPGKGVPGKGVPGKGVPGKGVPGKGVPGKGVPGKGVPGKGVPGRGVPGKGVPGKGVPGKGVPGKGVPGKGVPGKGVPGKGVPGKGVPGKGVPGVGVPGKGVPGKGVPGKGVPGKGVPGKGVPGKGVPGKGVPGKGVPGKGVPGVGVPGKGVPGKGVPGKGVPGKGVPGKGVPGKGVPGKGVPGKGVPGKGVPGIGVPGKGVPGKGVPGKGVPGKGVPGKGVPGKGVPGKGVPGKGVPGKGVPGVGVPGKGVPGKGVPGKGVPGKGVPGKGVPGKGVPGKGVPGKGVPGKGVPGVGVPGKGVPGKGVPGKGVPGKGVPGKGVPGKGVPGKGVPGKGVPGKGVPGAGVPGKGVPGKGVPGKGVPGKGVPGKGVPGKGVPGKGVPGKGVPGKGVPGVGVPGKGVPGKGVPGKGVPGKGVPGKGVPGKGVPGKGVPGKGVPGKGVPGVGVPGKGVPGKGVPGKGVPGKGVPGKGVPGKGVPGKGVPGKGVPGKG